European Patent Application EP 4 130 258 A1, published February 8, 2023. Title: Microorganisms with viral decoy receptors. Applicant: Evonik Operations GmbH. The sequence listing filed with the application follows.

SEQUENCE LISTING (20 sequences)

SEQ ID NO: 1 - DNA, 1547 bp, Bacillus subtilis
tcggagagtttgatcctggctcaggacgaacgctggcggcgtgcctaatacatgcaagtcgagcggacagatgggagcttgctccctgatgttagcggcggacgggtgagtaacacgtgggtaacctgcctgtaagactgggataactccgggaaaccggggctaataccggatggttgtttgaaccgcatggttcaaacataaaaggtggcttcggctaccacttacagatggacccgcggcgcattagctagttggtgaggtaatggctcaccaaggcaacgatgcgtagccgacctgagagggtgatcggccacactgggactgagacacggcccagactcctacgggaggcagcagtagggaatcttccgcaatggacgaaagtctgacggagcaacgccgcgtgagtgatgaaggttttcggatcgtaaagctctgttgttagggaagaacaagtaccgttcgaatagggcggtaccttgacggtacctaaccagaaagccacggctaactacgtgccagcagccgcggtaatacgtaggtggcaagcgttgtccggaattattgggcgtaaagggctcgcaggcggtttcttaagtctgatgtgaaagcccccggctcaaccggggagggtcattggaaactggggaacttgagtgcagaagaggagagtggaattccacgtgtagcggtgaaatgcgtagagatgtggaggaacaccagtggcgaaggcgactctctggtctgtaactgacgctgaggagcgaaagcgtggggagcgaacaggattagataccctggtagtccacgccgtaaacgatgagtgctaagtgttagggggtttccgccccttagtgctgcagctaacgcattaagcactccgcctggggagtacggtcgcaagactgaaactcaaaggaattgacgggggcccgcacaagcggtggagcatgtggtttaattcgaagcaacgcgaagaaccttaccaggtcttgacatcctctgacaatcctagagataggacgtccccttcgggggcagagtgacaggtggtgcatggttgtcgtcagctcgtgtcgtgagatgttgggttaagtcccgcaacgagcgcaacccttgatcttagttgccagcattcagttgggcactctaaggtgactgccggtgacaaaccggaggaaggtggggatgacgtcaaatcatcatgccccttatgacctgggctacacacgtgctacaatggacagaacaaagggcagcgaaaccgcgaggttaagccaatcccacaaatctgttctcagttcggatcgcagtctgcaactcgactgcgtgaagctggaatcgctagtaatcgcggatcagcatgccgcggtgaatacgttcccgggccttgtacacaccgcccgtcacaccacgagagtttgtaacacccgaagtcggtgaggtaaccttttaggagccagccgccgaaggtgggacagatgattggggtgaagtcgtaacaaggtagccgtatcggaaggtgcggctggatcacctccttt

SEQ ID NO: 2 - DNA, 1197 bp, Bacillus subtilis
gtgaaaaataaatggctgtcttttttttcgggtaaggtccagcttgaattgacgggaagagggattgagcggctccttaatgaatgcacaagacaggggattccggtctttcatgtcaaaaaaaagaaagaagccgtatcgttatatatacagcttcaggatgtacatgcctttcggcgggtgagaagtaaatttaaatgtaaagcccgatttatcaatcggaagggttttcccttcctgttgctgaaatcaaagctgaatatagggtttacgatcggttttgcgatttttttcatccttttgtttttgctgtccaatatggtgtggaaaattgatgtgacaggcgctaagcctgaaacagaacatcaaatgaggcagcatcttaatgaaatcggcgtcaaaaagggccgtctgcagtttttaatgatgtcgcccgaaaaaatacagaaatcattaaccaatggaatagacaatatcacttgggtcggagttgatctgaaggggacgaccattcacatgaaagtcgtggagaaaaatgagcccgaaaaagaaaagtatgttagcccgcgcaatattgtcgccaaaaagaaagcaacgattacgagaatgtttgtgcaaaaaggacagcccatggctgccatacacgatcatgttgaaaagggtcagctgcttgtttcggggctgatcggcagcgaagaccatcagcaggaagtcgcctcaaaagctgaaatttacggagaaacctggtatagatcagaagtgacagtcccgcttgaaacattatttaacgtctatacgggcaaagtaaggacaaagcacaagctttcttttggctcgttggcaatcccgatctgggggatgacgtttaaaaaagaggaattgaagcatccaaaaacagaacaagaaaagcattcgcttcattttctcggatttaagctccctgtatcctatgtcaaagagcaaacgagagaaagtgaagaggctttacgaaaatatacgaaagaagaagcagttcaagaaggcattaaattgggtaaacaggatgtagaggataaaataggcgaaaacggcgaggtgaaaagtgaaaaagttttgcaccagactgttgagaatggtaaagtaaagttgattattctctaccaagttatagaagatatcgttcaaaccacacctattgtcagggagactgaagaatga

SEQ ID NO: 3 - DNA, 1923 bp, Bacillus subtilis
gtggctatggaacagcagcaaaacagttatgatgaaaatcagatacaggtactagaaggattggaagctgttcgtaaaagaccggggatgtatatcggttcgacaaacagcaaaggccttcaccacctggtatgggaaattgtcgacaatagtattgacgaagccctcgccggttattgtacggatatcaatatccaaatcgaaaaagacaacagtatcacggttgtagataatggccgcggtattccagtcggtattcatgaaaaaatgggccgtcctgcggtagaagtcattatgacggtgcttcatgccggaggaaaatttgacggaagcggctataaagtatccggaggattacacggtgtaggtgcgtcggtcgtaaacgcactatcaacagagcttgatgtgacggttcaccgtgacggtaaaattcaccgccaaacctataaacgcggagttccggttacagaccttgaaatcattggcgaaacggatcatacaggaacgacgacacattttgtcccggaccctgaaattttctcagaaacaaccgagtatgattatgatctgcttgccaaccgcgtgcgtgaattagcctttttaacaaagggcgtaaacatcacgattgaggataaacgtgaaggacaagagcgcaaaaatgaataccattacgaaggcggaattaaaagttatgtagagtatttaaaccgctctaaagaggttgtccatgaagagccgatttacattgaaggcgaaaaggacggcattacggttgaagtggctttgcaatacaatgacagctacacaagcaacatttactcgtttacaaacaacattaatacgtacgaaggcggtacccatgaagctggcttcaaaacgggcctgactcgtgttatcaacgattacgccagaaaaaaagggcttattaaagaaaatgatccaaacctaagcggagatgacgtaagggaagggctgacagcgattatttcaatcaaacaccctgatccgcagtttgagggccaaacgaaaacaaagctgggcaactcagaagcacggacgatcaccgatacgttattttctacggcgatggaaacatttatgctggaaaatccagatgcggccaaaaaaattgtcgataaaggcttaatggcggcaagagcaagaatggctgcgaaaaaagcccgtgaactaacacgtcgtaagagtgctttggaaatttcaaacttgcccggtaagttagcggactgctcttcaaaagatccgagcatctccgagttatatatcgtagagggtgactctgccggaggatctgctaaacaaggacgcgacagacatttccaagccattttgccgcttagaggtaaaatcctaaacgttgaaaaggccagactggataaaatcctttctaacaacgaagttcgctctatgatcacagcgctcggcacaggtattggggaagacttcaaccttgagaaagcccgttaccacaaagttgtcattatgacagatgccgatgttgacggcgcgcacatcagaacacttctgttaacgttcttttacagatatatgcgccaaattatcgaaaatggctacgtgtacattgcgcagccgccgctctacaaggttcaacaggggaaacgcgttgaatatgcgtacaatgacaaggagcttgaagagctgttaaaaactcttcctcaaacgcctaagcctggactgcagcgttacaaaggtcttggtgaaatgaatgccacccagctatgggagacaaccatggatcctagctccagaacacttcttcaggtaactcttgaagatgcaatggatgcggacgagacttttgaaatgcttatgggcgacaaggtagaaccgcgccgaaacttcatagaagcgaatgcgagatacgttaaaaatcttgacatctaa

SEQ ID NO: 4 - DNA, 3582 bp, Bacillus subtilis
ttgacaggtcaactagttcagtatggacgacaccgccagcgcagaagctatgctcgcattagcgaagtgttagaattaccaaatctcattgaaattcaaacctcttcttatcagtggtttcttgatgagggtcttagagagatgtttcaagacatatcaccaattgaggatttcactggtaacctctctcttgagttcattgattatagtttaggtgagcctaaatatcctgtagaggaatcaaaagaacgtgatgtgacttactcagctccgctaagagtgaaggttcgtttaattaacaaagaaactggagaggtaaaagaccaagatgtcttcatgggtgatttccctattatgacagatacaggtacttttatcattaacggtgcggaacgtgttatcgtttcccagcttgttcggtctccaagtgtatatttcagtggtaaagtagacaaaaacggtaaaaaaggttttaccgcaactgtcattccaaaccgtggcgcatggttagaatacgaaactgatgcgaaagatgttgtttatgtccgcattgatcgcacacgtaagttgccggttacggttcttttgcgtgctctcggcttcggctccgatcaagagattcttgatctcataggagaaaacgaatacctgcgaaatacgcttgataaagataacacagaaaacagcgacaaagcgttactggaaatttacgagcgtctccgtcctggagagccgcctacagtagaaaatgcgaaaagcttgcttgattctcgtttctttgatccgaaacgatacgatcttgccaatgtaggacgctataaaattaataaaaaacttcatattaagaatcgcctcttcaatcagagacttgctgaaacgcttgttgatcctgaaacaggagaaatccttgctgaaaaaggtcagattcttgatagaagaacacttgataaagtactgccatacttagaaaacggaatcggtttcagaaagctgtatccgaatggtggcgttgttgaagatgaagtgactcttcaatcaattaaaatctttgctccgactgatcaagaaggagaacaggttattaatgtaatcggcaatgcttacatcgaagaagagattaaaaacatcacgcctgctgatattatttcttcaatcagctacttcttcaacctgctgcacggagtaggcgacacagatgatatcgatcatcttggaaaccgccgtttacgttctgtaggcgagcttctccagaatcaattccgtatcggtttaagccgtatggagcgtgtggttcgtgagagaatgtcaattcaagatacgaatacaattacgcctcagcaactgatcaatattcgtcctgttattgcgtccattaaagagttctttggaagctcacagctttctcaattcatggatcagacgaacccgcttgctgaattaacgcacaagcgtcgtctgtcagcattaggaccgggcggattgacacgtgagcgtgccggaatggaagtgcgtgacgttcactactcccactatggccgtatgtgtccgattgaaacgcctgagggcccgaacatcggtttgatcaactcactatcatcttatgcaaaagtaaaccgttttggctttattgaaacgccatatcgccgcgttgaccctgaaacagggaaggtaacgggcagaatcgattacttaactgctgatgaagaggataactatgttgtcgctcaagcgaatgctcgtcttgatgacgaaggcgcctttattgatgacagcatcgtagctcgtttccgtggggagaacaccgttgtttccagaaatcgtgtagactacatggatgtatcgcctaagcaggttgtatctgctgcgacagcatgtatcccgttcttagaaaacgatgactccaaccgtgccctcatgggagcgaacatgcagcgtcaggctgtgcctttgatgcagccggaagcgccatttgttggaactggtatggaatacgtatcaggaaaagactctggtgccgctgttatttgtaaacaccctggtatcgttgaacgcgtagaagcgaaaaacgtttgggttcgccgttatgaagaagtagacggtcaaaaagtaaaaggaaacctggataaatacagcctgctgaaatttgtccgctctaaccaaggtacgtgctacaaccagcgtccgatcgtaagtgtcggcgatgaagtggtaaaaggagaaatccttgctgacggtccttctatggagcttggtgaacttgcacttggccgtaacgtaatggtcggcttcatgacatgggatggctacaactatgaggatgccatcatcatgagtgaacgcctagtgaaggatgatgtttatacatctatccacattgaagaatacgaatcagaagcacgtgatacgaaacttggacctgaagaaatcactcgcgatattccaaacgtcggtgaagatgcgcttcgcaatcttgatgaccgcggaatcatccgtattggggcagaagtaaaagacggagatcttcttgttggtaaagtaacgcctaaaggcgtaactgaactgaccgcagaagaacgccttcttcacgccatctttggcgagaaagcccgcgaggttcgtgatacttctcttcgtgtgcctcatggcggcggcggaattatccatgacgttaaagtcttcaaccgtgaagacggagacgaacttcctccaggtgttaaccagttagtacgcgtatatatcgttcagaaacgtaagatttctgaaggggataaaatggccggtcgtcacggtaataaaggtgttatctctaagattcttcctgaagaggatatgccttaccttcctgacggcacaccaattgatatcatgcttaacccgctgggcgtaccatcacgtatgaacatcgggcaggtattggaacttcacatgggtatggccgctcgttaccttggcattcacattgcatctcctgtatttgacggagcgcgagaagaggatgtctgggaaacacttgaagaagccggcatgtctcgtgacgccaaaacagtgctttacgacggacgtactggagagccgtttgataaccgtgtatctgtcggtatcatgtacatgatcaaactagctcacatggttgacgataaacttcatgcacgctctacaggcccttactcacttgttacgcagcagcctcttggcggtaaagcgcaatttggcggacagcgttttggtgagatggaggtttgggcacttgaagcttacggtgcggcttacactcttcaagaaattctgactgttaagtctgatgacgtggttggacgtgtgaaaacatacgaagccatcgttaaaggcgacaatgttcctgaaccaggtgttccggaatcattcaaagtattaatcaaagaacttcaaagcttaggtatggatgtcaaaatcctttctggtgatgaagaagaaatagaaatgagagatttagaagacgaagaagatgcgaaacaagctgacggcctggcattatcaggtgatgaagagccggaagaaacagcatctgcagacgttgaacgcgatgtagtaacaaaagaataa

SEQ ID NO: 5 - DNA, 1632 bp, Bacillus subtilis
atggcaaaagaaattaagtttagtgaagaagctcgccgcgcaatgcttcgcggtgtcgatgcacttgctgatgctgttaaagtaactttaggaccaaaaggacgcaacgtggttctagagaaaaaattcggttctccgttaatcacaaatgacggtgtaacaatcgctaaagaaatcgagctagaagacgcgtttgaaaacatgggtgctaagcttgttgctgaagtagccagcaaaacaaacgacgttgccggtgacggtacaacaactgcaacagttcttgcgcaagcaatgatccgtgaaggccttaaaaacgtaacagcaggcgctaaccctgtaggcgtgcgtaaagggatggaacaagctgtagcggttgcgatcgaaaacttaaaagaaatttctaagccaatcgaaggcaaagagtctatcgctcaggttgctgcgatctctgctgctgatgaggaagtcggaagccttatcgctgaagcaatggagcgcgtaggaaacgacggcgttatcacaatcgaagagtctaaaggcttcacaactgagcttgaagttgttgaaggtatgcaattcgaccgcggatatgcgtctccttacatggtaactgactctgataagatggaagcggttcttgacaatccttacatcttaatcacagacaaaaaaatcacaaacattcaagaaatccttcctgtgcttgagcaggttgttcagcaaggcaaaccattgcttttgatcgcagaagacgttgaaggcgaagcacttgcaacacttgttgtgaacaaacttcgcggcacattcaacgcagttgctgttaaagctcctggcttcggtgaccgccgtaaagcaatgcttgaagacatcgctgtccttactggcggagaagtcatcacagaagatcttggccttgacctgaaatctactcaaatcgctcaattgggacgcgcttctaaagttgtcgttactaaagaaaacacaacaatcgttgaaggcgctggcgaaacagacaaaatttctgcccgcgtgactcaaatccgcgctcaagtagaagaaacaacttctgaattcgacagagaaaaattacaagagcgtcttgcgaaacttgctggcggcgtagctgtcatcaaagtcggagctgcgactgaaactgagctgaaagagcgtaaacttcgcatcgaagacgccttgaactcaactcgcgcagctgttgaagaaggcatcgtatccggtggtggtacagcgcttgtaaacgtatataacaaagtcgctgcagttgaagctgaaggcgatgcgcaaacaggtatcaacatcgtgcttcgcgcgcttgaagagccaatccgtcaaatcgcacataacgctggtcttgaaggatctgtcatcgttgagcgcctcaaaaacgaagaaatcggcgtaggcttcaacgctgcaactggcgaatgggtaaacatgatcgaaaaaggtatcgttgacccaacaaaagttacacgctcagctcttcaaaacgctgcgtctgtagctgcaatgttcttaacaactgaagccgttgtcgctgacaagccggaagaaaacgctggcggcggaatgcctgacatgggcggcatgggcggtatgggcggcatgatgtaa

SEQ ID NO: 6 - DNA, 1547 bp, Bacillus subtilis
tcggagagtttgatcctggctcaggacgaacgctggcggcgtgcctaatacatgcaagtcgagcggacagatgggagcttgctccctgatgttagcggcggacgggtgagtaacacgtgggtaacctgcctgtaagactgggataactccgggaaaccggggctaataccggatggttgtttgaaccgcatggttcaaacataaaaggtggcttcggctaccacttacagatggacccgcggcgcattagctagttggtgaggtaacggctcaccaaggcaacgatgcgtagccgacctgagagggtgatcggccacactgggactgagacacggcccagactcctacgggaggcagcagtagggaatcttccgcaatggacgaaagtctgacggagcaacgccgcgtgagtgatgaaggttttcggatcgtaaagctctgttgttagggaagaacaagtaccgttcgaatagggcggtaccttgacggtacctaaccagaaagccacggctaactacgtgccagcagccgcggtaatacgtaggtggcaagcgttgtccggaattattgggcgtaaagggctcgcaggcggtttcttaagtctgatgtgaaagcccccggctcaaccggggagggtcattggaaactggggaacttgagtgcagaagaggagagtggaattccacgtgtagcggtgaaatgcgtagagatgtggaggaacaccagtggcgaaggcgactctctggtctgtaactgacgctgaggagcgaaagcgtggggagcgaacaggattagataccctggtagtccacgccgtaaacgatgagtgctaagtgttagggggtttccgccccttagtgctgcagctaacgcattaagcactccgcctggggagtacggtcgcaagactgaaactcaaaggaattgacgggggcccgcacaagcggtggagcatgtggtttaattcgaagcaacgcgaagaaccttaccaggtcttgacatcctctgacaatcctagagataggacgtccccttcgggggcagagtgacaggtggtgcatggttgtcgtcagctcgtgtcgtgagatgttgggttaagtcccgcaacgagcgcaacccttgatcttagttgccagcattcagttgggcactctaaggtgactgccggtgacaaaccggaggaaggtggggatgacgtcaaatcatcatgccccttatgacctgggctacacacgtgctacaatggacagaacaaagggcagcgaaaccgcgaggttaagccaatcccacaaatctgttctcagttcggatcgcagtctgcaactcgactgcgtgaagctggaatcgctagtaatcgcggatcagcatgccgcggtgaatacgttcccgggccttgtacacaccgcccgtcacaccacgagagtttgtaacacccgaagtcggtgaggtaaccttttaggagccagccgccgaaggtgggacagatgattggggtgaagtcgtaacaaggtagccgtatcggaaggtgcggctggatcacctccttt

SEQ ID NO: 7 - DNA, 1197 bp, Bacillus subtilis
gtgaaaaataaatggctgtcttttttttcgggtaaggtccagcttgaattgacgggaagagggattgagcggctccttaatgaatgcacaagacaggggattccggtctttcatgtcaaaaaaaagaaagaagccgtatcgttatatatacagcttcaggatgtacatgcctttcggcgggtaagaagtaaatttaaatgtaaagcccgatttatcaatcggaagggatttcccttcctgttgctgaaatcaaagctgaatatagggtttacgatcggttttgcgatttttttcattcttttgtttttgctgtccaatatggtgtggaaaattgatgtgacaggcgctaagcctgaaacagaacatcaaatgaggcagcatcttaatgaaatcggcgtcaaaaagggccgtctgcagtttttaatgatgtcgcccgaaaaaatacagaaatcattaaccaatggaatagacaatatcacttgggtcggagttgatctgaaggggacgaccattcatatgaaagttgtggagaaaaatgagcccgaaaaagaaaaatatgttagcccgcgcaatattgtcgccaaaaagaaagcaaccattacgagaatgtttgtgcaaaaaggacagcccatggccgccatacacgatcatgttgaaaagggacagctgcttgtttcgggactgatcggcagcgaagaccatcagcaggaagtcgcctcaaaagcagaaatttatggagaaacctggtatagatcagaagtgacagtcccgcttgaaacattatttaacgtctatacgggcaaagtaaggacaaagcacaagctttcttttggttctttggcaatcccgatctgggggatgacgtttaaaaaagaggaattgaagcatccaaaaacagaacaagaaaagcattcgcttcattttctcggatttaagctccctgtatcctatgtcaaagagcaaacgagagaaagtgaagaggctttgcgaaaatatacaaaagaagaagcagttcaagaaggcattaaattgggtaaacaggatgtagaggataaaataggcgaaaacggcgaggtgaaaagtgaaaaagttttgcaccagactgttgagaatggtaaagtaaagttgattattctctaccaagttatagaagatatcgttcaaaccacacctattgtcagggagactgaagaatga

SEQ ID NO: 8 - DNA, 1923 bp, Bacillus subtilis
gtggctatggaacagcagcaaaacagttatgatgaaaatcagatacaggtactagaaggattggaagctgttcgtaaaagaccggggatgtatatcggttcgacaaacagcaaaggccttcaccacttggtatgggaaattgtcgacaatagtattgacgaagccctcgccggttattgtacggatatcaatatccaaatcgaaaaagacaacagtatcacggttgtagataatggccgcggtattccagtcggtattcatgaaaaaatgggccgtcctgcggtagaagtcattatgacggtgcttcatgccggaggaaaatttgacggaagcggctataaagtatccggaggattacacggtgtaggtgcgtcggtcgtaaacgcactatcaacagagcttgatgtgacggttcaccgtgacggtaaaattcaccgccaaacctataaacgcggagttccggttacagaccttgaaatcattggcgaaacggatcatacaggaacgacgacacattttgtcccggaccctgaaattttctcagaaacaaccgagtatgattacgatctgcttgccaaccgcgtgcgtgaattagcctttttaacaaagggcgtaaacatcacgattgaagataaacgtgaaggacaagagcgcaaaaatgaataccattacgaaggcggaattaaaagttatgtagagtatttaaaccgctctaaagaggttgtccatgaagagccgatttacattgaaggcgaaaaggacggcattacggttgaagtggctttgcaatacaatgacagctacacaagcaacatttactcgtttacaaacaacattaacacgtacgaaggcggtacccatgaagctggcttcaaaacgggcctgactcgtgttatcaacgattacgccagaaaaaaagggcttattaaagaaaatgatccaaacctaagcggagatgacgtaagggaagggctgacagcgattatttcaatcaaacaccctgatccgcagtttgagggccaaacaaaaacaaagctgggcaactcagaagcacggacgatcaccgatacgttattttctacggcgatggaaacatttatgctggaaaatccagatgcagccaaaaaaattgtcgataaaggtttaatggcggcaagagcaagaatggctgcgaaaaaagcgcgtgaactaacacgccgtaagagtgctttggaaatttcaaacctgcccggtaagttagcggactgctcttcaaaagatccgagcatctccgagttatatatcgtagagggtgactctgccggaggatctgctaaacaaggacgcgacagacatttccaagccattttgccgcttagaggtaaaatcctaaacgttgaaaaggccagactggataaaatcctttctaacaacgaagttcgctctatgatcacagcgctcggcacaggtatcggagaagacttcaaccttgagaaagcccgttaccacaaagttgtcattatgacagatgccgatgttgacggcgcgcacatcagaacactgctgttaacgttcttttacagatatatgcgccaaattatcgaaaatggctacgtgtacattgcgcagccgccgctctacaaggttcaacaggggaaacgcgttgaatatgcatacaatgacaaggagcttgaagagctgttaaaaactcttcctcaaacgcctaagcctggactgcagcgttacaaaggtcttggtgaaatgaatgccacccagctatgggagacaaccatggatcctagctccagaacacttcttcaggtaactcttgaagatgcaatggatgcggatgagacttttgaaatgcttatgggcgacaaggtagaaccgcgccgaaacttcatagaagcgaatgcgagatacgttaaaaatcttgacatctaa

SEQ ID NO: 9 - DNA, 3582 bp, Bacillus subtilis
ttgacaggtcaactagttcagtatggacgacaccgccagcgcagaagctatgctcgcattagcgaagtgttagaattaccaaatctcattgaaattcaaacctcttcttatcagtggtttcttgatgagggtcttagagagatgtttcaagacatatcaccaattgaggatttcactggtaacctctctcttgagttcattgattatagtttaggtgagcctaaatatcctgtagaggaatcaaaagaacgtgatgtgacttactcagctccgctaagagtgaaggttcgtttaattaacaaagaaactggagaggtaaaagaccaagatgtcttcatgggtgatttccctattatgacagatacaggtacttttatcattaacggtgcggaacgtgttatcgtttcccagcttgttcggtctccaagtgtatatttcagtggtaaagtagacaaaaacggtaaaaaaggttttaccgcaactgtcattccaaaccgtggcgcatggttagaatacgaaactgatgcgaaagatgttgtttatgtccgcattgatcgcacacgtaagttgccggttacggttcttttgcgtgctctcggcttcggctccgatcaagagattcttgatctcataggagaaaacgaatacctgcgaaatacgcttgataaagataacacagaaaacagcgacaaagcgttgctggaaatttacgagcgtctccgtcctggagagccgcctacagtagaaaatgcgaaaagcttgcttgattctcgtttctttgatccgaaacgatacgatcttgccaatgtaggacgctataaaattaataaaaaacttcatattaagaatcgcctcttcaatcagagacttgctgaaacgcttgttgatcctgaaacaggagaaatccttgctgaaaaaggccagattcttgatagaagaacgcttgataaagtactgccatacttagaaaacggaatcggttttagaaagctgtatccgaatggcggcgttgttgaagatgaagtgactcttcaatcaattaaaatctttgctccgactgatcaagaaggagaacaggttatcaatgtaatcggcaatgcttacatcgaagaagagattaaaaacatcacgcctgctgatattatttcttcaatcagctacttcttcaacctgctgcacggagtaggcgacacagatgatatcgatcatcttggaaaccgccgtttacgttctgtaggcgagcttctccagaaccaattccgtatcggtttaagccgtatggagcgtgtggttcgtgagagaatgtcaattcaagatacgaatacaattacgcctcagcagctgatcaatattcgtcctgttattgcgtccattaaagagttctttggaagctcacagctttctcaattcatggatcagacgaacccgcttgctgaattaacgcacaagcgtcgtctgtcagcattaggaccgggcggattgacacgtgagcgtgccggaatggaagtgcgtgacgttcactactcccactatggccgtatgtgtccgattgaaacgcctgagggcccgaacatcggtttgatcaactcactatcatcttatgcaaaagtaaaccgttttggctttattgaaacgccatatcgccgcgttgaccctgaaacagggaaggtaacgggcagaatcgattacttaactgctgatgaagaggataactatgttgtcgctcaagcgaatgctcgtcttgatgacgaaggcgcctttattgatgacagcatcgtagctcgtttccgcggggagaacaccgttgtttccagaaatcgtgtagactacatggatgtatcgcctaagcaggttgtatctgctgcgacagcatgtatcccgttcttagaaaacgatgactccaaccgtgccctcatgggagcgaacatgcagcgtcaggctgtgcctttgatgcagccggaagcgccatttgttggaactggtatggaatacgtatcaggaaaagactctggtgccgctgttatttgtaaacaccctggtatcgttgaacgcgtagaagccaaaaacgtttgggttcgccgttatgaagaagtagacggtcaaaaagtaaaaggaaacctggataaatacagcctgctgaaatttgtccgctctaaccaaggtacgtgctacaaccagcgtccgatcgtaagtgtcggcgatgaagtggtaaaaggagaaatccttgctgacggtccttctatggagcttggtgaacttgcacttggccgtaacgtaatggtcggcttcatgacgtgggatggctacaactatgaggatgccatcatcatgagtgaacgcctagtgaaggatgatgtttatacatctatccacattgaagaatacgaatcagaagcacgtgatacgaaacttggacctgaagaaatcactcgcgatattccaaacgtcggtgaagatgcgcttcgcaatcttgatgaccgcggaatcatccgtattggggcagaagtaaaagacggagatcttcttgttggtaaagtaacgcctaaaggcgtaactgaactgactgccgaagaacgccttcttcacgccatctttggcgagaaagcccgcgaggttcgtgatacttctcttcgtgtgcctcatggcggcggcggaattatccatgacgttaaagtcttcaaccgtgaagacggagacgaacttcctccaggtgttaaccagttagtacgcgtatatatcgttcagaaacgtaagatttctgaaggggataaaatggccggtcgtcacggtaacaaaggtgttatctctaagattcttcctgaagaggatatgccttaccttcctgacggcacaccaattgatatcatgcttaacccgctgggcgtaccatcacgtatgaacatcgggcaggtattggaacttcacatgggtatggccgctcgttaccttggcattcacattgcatctcctgtatttgacggagcgcgagaagaggatgtctgggaaacacttgaagaagccggcatgtctcgtgacgccaaaacagtgctttacgacggacgtactggagagccgtttgataaccgtgtatctgtcggtatcatgtacatgatcaaactggctcacatggttgacgataaacttcatgcacgctctacaggcccttactcacttgttacgcagcagcctcttggcggtaaagcgcaatttggcggacagcgttttggtgagatggaggtttgggcacttgaagcttacggtgcggcttacactcttcaagaaattctgactgttaagtctgatgacgtggttggacgtgtgaaaacatacgaagccatcgttaaaggcgacaatgttcctgaaccaggtgttccggaatcattcaaagtattaatcaaagaacttcaaagcttaggtatggatgtcaaaatcctttctggtgatgaagaagaaatagaaatgagagatttagaagacgaagaagatgcgaaacaagctgacggcctggcattatcaggtgatgaagagccggaagaaacagcatctgcagacgttgaacgcgatgtagtaacaaaagaataa

SEQ ID NO: 10 - DNA, 1635 bp, Bacillus subtilis
atggcaaaagaaattaagtttagtgaagaagctcgccgcgcaatgcttcgcggtgtcgatgcacttgctgatgctgttaaagtaactttaggaccaaaaggacgcaacgtggttctagagaaaaaattcggttctccgttaatcacaaatgacggtgtaacaatcgctaaagaaatcgagctagaagacgcgtttgaaaacatgggtgctaagcttgttgctgaagtagccagcaaaacaaacgacgttgccggtgacggtacaacaactgcaacagttcttgcgcaagcaatgatccgtgaaggccttaaaaacgtaacagcaggcgctaaccctgtaggcgtgcgtaaagggatggaacaagctgtagcggttgcgatcgaaaacttaaaagaaatttctaagccaatcgaaggcaaagagtctatcgctcaggttgctgcgatctctgctgctgatgaggaagtcggaagccttatcgctgaagcaatggagcgcgtaggaaacgacggcgttatcacaatcgaagagtctaaaggcttcacaactgagcttgaagttgttgaaggtatgcaattcgaccgcggatatgcgtctccttacatggtaactgactctgataagatggaagcggttcttgacaatccttacatcttaatcacagacaaaaaaatcacaaacattcaagaaatccttcctgtgcttgagcaggttgttcagcaaggcaaaccattgcttctgatcgctgaggatgttgaaggcgaagcacttgctacacttgttgtgaacaaacttcgcggcacattcaacgcagtggctgttaaagctcctggtttcggtgatcgccgtaaagcaatgcttgaagacatcgctgtccttactggcggagaagtcatcacagaagatcttggccttgacctgaaatctactcaaatcgctcaattgggacgcgcttctaaagttgtcgttactaaagaaaacacaacaatcgttgaaggcgctggcgaaacagacaaaatttctgcccgtgtgactcaaatccgcgctcaagtggaagaaacaacttctgaattcgacagagaaaaattacaagagcgtcttgctaaacttgctggcggcgtagctgtcatcaaagtcggcgctgcgactgaaactgagctgaaagagcgtaaacttcgcatcgaagacgccttgaactcaactcgcgcagctgttgaagaaggcatcgtatccggtggtggtacagcgcttgtaaacgtatataacaaagtcgctgcagttgaagctgaaggcgatgctcaaacaggtatcaacatcgtgcttcgcgcgcttgaagagccaatccgtcaaatcgcacacaacgctggccttgaaggatctgtcatcgttgagcgcctcaaaaacgaagaaatcggcgtaggcttcaacgctgcaactggcgaatgggtaaacatgatcgaaaaaggtatcgttgacccaacaaaagttacacgctcagctcttcaaaacgctgcgtctgtagctgcaatgttcttaacaacagaagctgttgtcgctgacaagccagaagaaaacggtggcggcgcaggaatgcctgatatgggcggcatgggcggtatgggtggaatgatgtaa

SEQ ID NO: 11 - DNA, 1547 bp, Bacillus velezensis
tcggagagtttgatcctggctcaggacgaacgctggcggcgtgcctaatacatgcaagtcgagcggacagatgggagcttgctccctgatgttagcggcggacgggtgagtaacacgtgggtaacctgcctgtaagactgggataactccgggaaaccggggctaataccggatggttgtttgaaccgcatggttcagacataaaaggtggcttcggctaccacttacagatggacccgcggcgcattagctagttggtgaggtaacggctcaccaaggcaacgatgcgtagccgacctgagagggtgatcggccacactgggactgagacacggcccagactcctacgggaggcagcagtagggaatcttccgcaatggacgaaagtctgacggagcaacgccgcgtgagtgatgaaggttttcggatcgtaaagctctgttgttagggaagaacaagtgccgttcaaatagggcggcaccttgacggtacctaaccagaaagccacggctaactacgtgccagcagccgcggtaatacgtaggtggcaagcgttgtccggaattattgggcgtaaagggctcgcaggcggtttcttaagtctgatgtgaaagcccccggctcaaccggggagggtcattggaaactggggaacttgagtgcagaagaggagagtggaattccacgtgtagcggtgaaatgcgtagagatgtggaggaacaccagtggcgaaggcgactctctggtctgtaactgacgctgaggagcgaaagcgtggggagcgaacaggattagataccctggtagtccacgccgtaaacgatgagtgctaagtgttagggggtttccgccccttagtgctgcagctaacgcattaagcactccgcctggggagtacggtcgcaagactgaaactcaaaggaattgacgggggcccgcacaagcggtggagcatgtggtttaattcgaagcaacgcgaagaaccttaccaggtcttgacatcctctgacaatcctagagataggacgtccccttcgggggcagagtgacaggtggtgcatggttgtcgtcagctcgtgtcgtgagatgttgggttaagtcccgcaacgagcgcaacccttgatcttagttgccagcattcagttgggcactctaaggtgactgccggtgacaaaccggaggaaggtggggatgacgtcaaatcatcatgccccttatgacctgggctacacacgtgctacaatggacagaacaaagggcagcgaaaccgcgaggttaagccaatcccacaaatctgttctcagttcggatcgcagtctgcaactcgactgcgtgaagctggaatcgctagtaatcgcggatcagcatgccgcggtgaatacgttcccgggccttgtacacaccgcccgtcacaccacgagagtttgtaacacccgaagtcggtgaggtaaccttttaggagccagccgccgaaggtgggacagatgattggggtgaagtcgtaacaaggtagccgtatcggaaggtgcggctggatcacctccttt

SEQ ID NO: 12 - DNA, 1185 bp, Bacillus velezensis
gtgaaaaacaaatggctgtcatttttttcgggtaaagtccaagtagaagtcaaaggaaaagggattgaacggctgctgaatgaatgcacgagaaacggaatcgccatctttgcggtgaaaaaaaagcaagactgtgtcctgctgatgattcagcttcaggatgtacatgctttcagaagagtcatcagaaaacatgaatgcaaagcaagctttacaaaaagaaagggtcttccctttctgcttctcaaatcaaaattaaacctgggcttcactgcgggatttgtgatattttttgttatattatttcttttgtccaacatgatttgggaaattgatattaaaggggccaagcccgaaaccgagcatcagatggtaaagcaccttgaagaaatcggtgtgaaaaaaggccgtttgcaatttttaatgatgacgccggagaaaattcaaaaatcattaacaaacggtatcgataatattacgtgggtcggtgtggaattgaacgggacagcccttcatatgaaagtggtcgaaaaaaacgaaccgacaaaagaaaagtacgtgagcccccgccatatcgttgccaaaaagaaggcggtcatcaaaaggatgttcgtgcaaaaggggcagccgatggcttttgtgaacgatcatgttgacaaaggacagctcctcgtctcaggactgatcggaaatgaagaccggaaagtcgcctcaaaagcggaaatttacggagaaacatggtacaagtcagaagtaaccgtgcctcttgaaacatcatttacgctatatacgggtaaagtaaggacgaagcacaagctgtctttcggatcatggggcgtgcctttttggggctttgaatttaatgagaagccgctgaaacagccgaaaacagaggaagaaaagcatccgtttcaatttctggggatgaagcttccggtttcttacgttcaagaacagacaagagaaagtgaaacatccgtgcggacttatacgaaaggcgaagcggttcaggccggtatcaaaatgggaagacaagatgtagaaaagcgattaaacggcagcggagaggtggaaagtgaaaaagttttgcaccaatccgttgagaatggtaaagtaaagttgattattctctaccaagttatagaagatatcgttcaaaccacacctattgttcagggagactaa

SEQ ID NO: 13 - DNA, 1923 bp, Bacillus velezensis
atggctatggaacagcagcaaaatagttatgatgagaatcagatacaggtattagaaggtttggaagctgttcgaaagagaccggggatgtacatcggatcaactaacagcaaaggccttcaccacttggtgtgggaaatcgtcgacaacagtattgacgaggccctggccggttattgtacagatattaatatcgagattgaaaaagataacagcattaccgttaaggacaacgggcgcggaattccggtcggtatccaggagaagatgggccgccctgcggttgaagtcatcatgaccgttctccacgccggcggtaaatttgacggaagcggatataaagtatccggcggtcttcacggtgtaggggcgtccgtcgtaaacgccttgtcgaccactcttgacgttacggttcatcgtgacggaaaaatccactatcaggcgtacgagcgcggtgtgcctgtggccgatcttgaagtgatcggtgatactgataagaccggaacgattacgcacttcgttccggatccggaaatcttcaaagaaacaactgtatacgactatgatctgctttcaaaccgtgtccgggaattggccttcctgacaaaaggcgtaaacatcacgattgaagacaaacgtgaaggacaagaacggaaaaacgagtaccactacgaaggcggaatcaaaagctatgttgagtacttaaaccgttccaaagaagtcgttcatgaagagccgatttatatcgaaggcgagaaagacggcataacggttgaagttgcattgcaatacaacgacagctatacaagcaatatttattctttcacaaataatatcaacacatacgaaggcgggacgcacgaggccggatttaaaactggtctgacccgtgtcataaacgactatgcaagaagaaaagggattttcaaagaaaatgatccgaatttaagcggggatgatgtgagagaagggctgactgccattatttcaattaagcaccctgatccgcaattcgaagggcagacgaaaaccaagctcggcaactctgaagcgagaacgatcactgacacgctgttttcttctgcgctggaaacattccttcttgaaaatccggactcagcccgcaaaatcgttgaaaaaggtttaatggccgcaagagcgcggatggcagcgaaaaaagcgcgggaattgacccggcgcaaaagtgcgcttgagatttccaatctgccgggcaaactggcggactgttcttctaaagatccgagcatttccgagctgtatatcgtagagggtgactctgcgggcggatcagcgaaacagggacgggaccgtcatttccaagccattctgccgctgcgcggtaagattctgaacgttgagaaagccagacttgataagattctctcaaacaatgaggtcagatcaatgatcacggccctcggaacaggaatcggcgaagattttaatcttgaaaaagcgcgttatcataaagtggtcatcatgacggatgccgatgttgacggcgcccacatcagaacgcttttattaacgttcttctacagatacatgcgggaaatcatcgaaaacggctatgtctacattgcccagccgccgctttataaagtgcagcagggaaaacgggtggaatacgcttataacgataagcagcttgatgagctgttaaaagagcttccgcaatcacctaagcccggcctccagcgttataaaggtcttggagaaatgaacgcgactcagctttgggaaacgacaatggaccctgcgaccagaacgcttctgcaagtcaatcttgaagatgcaatggacgctgacgagacttttgaaatgctgatgggtgacaaagtagaaccgcggagaaacttcatagaagcaaacgccagatacgtgaaaaatcttgatatttaa

SEQ ID NO: 14 - DNA, 3582 bp, Bacillus velezensis
ttgacaggtcaactagttcagtatggacgacaccgccagcgcagaagctatgctcgcattagcgaagtgttagaattaccaaatctcattgaaattcaaacctcttcttatcagtggtttcttgatgagggtcttagagagatgtttcaagacatatcaccaattgaggatttcactggtaacctctctcttgagttcattgattatagtttaggtgagcctaaatatcctgtagaggaatcaaaagaacgtgatgtgacttactcagctccgctaagagtgaaggttcgtttaattaacaaagaaactggagaggtaaaagaccaagatgtcttcatgggtgatttccctattatgacagatacaggtacttttatcattaacggtgcagaacgtgttatcgtatctcagcttgttcggtctccaagtgtatatttcagtggtaaagtagacaaaaacggtaaaaaaggttttaccgcgactgtcattccaaaccgtggcgcatggttagaatacgaaactgatgcgaaagatgttgtgtatgtccgcattgatcgcacacgtaagttgccggttacggttcttttgcgtgctctcggcttcggttccgaccaagagattctcgatctcattggtgagaacgaatatctccgcaatacactggataaggacaacactgaaaacagtgacaaagcgcttcttgaaatctatgagcgccttcgtcccggagagccgcctacagtagaaaacgcaaaaagcttgctggattcccgtttcttcgatccgaagcgatacgaccttgcgaatgtaggacgctataaaattaataaaaagcttcatatcaagaaccgcctgtttaaccagcgacttgcagaaacactggtggatccggaaaccggtgaaattctcgctgaaaaagggcagattcttgacagaagaacacttgataaagtactgccatacttagaaaatggaatcggcttcagaaaactttatcctaacggcggcgtcgtcgaggatgaagtgatgcttcaatccattaaaatctatgctcctaccgatgcagaaggagagcagacgatcaatgtgatcggcaatgcttacatcgaagaggcgattaaaaacattacgcctgctgatattatttcttctatcagctacttcttcaacctcctgcacggagtgggcgacactgatgatatcgaccatctcggaaaccgccgtctgcgttctgtaggtgagctcctgcaaaaccaattccgtatcggtttaagccggatggaacgtgtcgtacgtgaaagaatgtctattcaagacacaaatacaatcacgccgcagcagctgattaacatcagacctgttattgcgtctattaaagagttcttcggaagctcacagctttctcaattcatggatcagacgaacccgcttgctgaattgacgcacaaacgccgtctgtcagctctcggaccgggcggtttgacacgtgagcgcgcaggtatggaagtacgtgacgttcactactctcactatggccgtatgtgtccgattgaaacgcctgagggcccgaacatcggtttgatcaactcattgtcatcatttgcgaaagtaaaccgctttggtttcattgagacgccataccgccgcgttgatcctgaaacaggaaaagtaacgcctagaatcgactacctgactgctgatgaagaggataactatgtcgtagcccaagcgaatgctaagctgagcgatgacggttctttcttggatgacagcatcgtagcgcgtttcagaggggaaaacaccgttgtagcccgcaaccgcgtggattacatggacgtatctcctaaacaggttgtttctgctgcgacagcatgtattccgttcttggaaaacgatgactcgaaccgcgccctcatgggagcgaacatgcagcgtcaggctgtgcctttgatgcagccggaagctccgatcgtcggaacgggtatggaatacgtatccggtaaagactccggtgcagccgttatttgtaaacaccctggtatcgttgaacgggtggaagcgaaaaacgtatgggtgcgccgctatgaagaaattgacggccaaaaagtaaaaggcaacctggataagtacagcttgctgaaatttgtccgctccaaccaaggtacgtgctacaaccagcgtccgatcgtcagtgtcggcgatgaagtagtcaaaggagaaatccttgctgacggaccttcaatggagcttggtgaacttgctctcggccgcaacgtaatggtcggcttcatgacatgggatggttacaactatgaggatgccatcatcatgagtgaacgccttgtgaaagatgatgtatacacatctattcacattgaagaatatgaatcagaagcacgtgatacaaagcttgggccggaagagatcacccgcgatattccaaacgtaggggaagacgcgcttcgcaatcttgatgaccgcggaattatccgtatcggtgcggaagtcaacgacggagaccttctcgtaggtaaagtaacgcctaaaggtgtaactgagcttacggctgaagaacgccttctgcatgcgatctttggagaaaaagcgcgtgaagtccgtgatacttctctccgtgtgcctcacggcggcggcggaattatccacgacgtaaaagtcttcaaccgtgaagacggcgacgaacttcctccgggagtgaaccagcttgtacgcgtatatatcgttcagaaacgtaagatttctgaaggtgataaaatggccggacgtcacggaaacaaaggggttatctcgaagattcttcctgaagaagatatgccttaccttcctgacggcacgccgatcgatatcatgcttaacccgctgggtgtaccatcacgtatgaatatcggtcaggtattagaacttcacatgggtatggctgcccgctacctcggcattcacatcgcgtcacctgtatttgacggcgcgcgtgaagaagatgtgtgggaaacacttgaagaagcaggcatgtcaagagacgctaaaacagttctttatgacggccgtacgggagaaccgttcgacaaccgtgtatcagtcggaatcatgtacatgatcaaactggcgcacatggttgatgataaacttcatgcccgttctacaggtccttactcacttgttacgcagcagcctctcggcggtaaagcccaattcggcggacagcgtttcggtgagatggaggtttgggcgcttgaagcttacggcgcagcttacacgcttcaagaaatcctgactgtgaagtccgatgacgtggtcggacgtgtgaaaacatatgaagccatcgtcaaaggcgacaatgttccagagcctggtgttccggaatcattcaaagtattgatcaaagagcttcaaagcttaggtatggacgtaaaaatcctttcaggcgatgaagaagaaatagaaatgagagatctagaagacgaggaagatgcgaaacaggctgacggccttgcattatcaggtgatgaagcgccggaagaaacagcatctccagacgttgaacgtgacgcagtaacgaaagaatag

SEQ ID NO: 15 - DNA, 1635 bp, Bacillus velezensis
atggcaaaagatattaagtttagtgaagaagcacgccgcgctatgcttcgcggtgtcgatgcgcttgctgacgctgtaaaagtaactttagggccaaaaggacgcaacgtggttctggagaaaaaattcggttctccgttaattacaaatgacggtgtgacaatcgcaaaagaaattgaacttgaagatgcgtttgaaaacatgggtgcgaagcttgtagctgaagtagccagcaaaacaaacgacgttgccggtgacggtacgacgactgcgactgtacttgcgcaggctatgatccgcgaaggcttgaaaaacgtaactgcgggggctaaccctgtcggcgtgcgtaaaggtatggaacaagctgtaaccgttgcaatcgaaaacttaaaagaaatttctaagccgatcgaaggcaaagagtctatcgctcaggttgctgcgatctctgctgctgatgaggaagtcggaagccttatcgctgaagcaatggagcgcgtaggaaacgacggcgtcatcacaatcgaagagtctaaaggtttcacaactgagcttgaagttgtggaaggtatgcaattcgaccgcggatatgcgtctccttacatggtgactgactctgataagatggaagcggttcttgacaatccttacatcttaatcacagacaaaaaaatcacaaacattcaagaaatccttcctgtgcttgagcaagttgtacagcaaggcaaaccattgcttctgatcgctgaagatgttgaaggtgaagctcttgctacactcgttgtcaacaaacttcgcggcacattcaacgctgttgccgttaaagctcctggcttcggtgaccgccgtaaagcaatgcttgaagacatctctgttcttacaggcggagaagtaatcacagaagacttaggccttgacctgaaatctactgaaatcggacaattgggacgcgcttctaaagttgtggtaacgaaagaaaacacaacaatcgtagaaggcgccggcgatactgaaaaaatcgctgcacgcgtcaaccaaatccgcgctcaagtggaagaaacaacttctgaattcgacagagaaaaattacaagagcgtcttgcgaaacttgccggcggcgtagctgtcatcaaagtcggcgctgcgactgaaactgagctgaaagagcgtaaacttcgcattgaagatgccctcaactcaactcgcgcagctgttgaagaaggcatcgtatccggcggtggtacagcgcttgtcaacgtatacaacaaagtcgctgcagttgaagctgaaggcgatgcgcaaacaggtatcaacatcgtgcttcgcgcgcttgaagagccgatccgtcaaatcgcgcacaatgcaggtcttgaaggatctgtcatcgttgagcgcctgaaaaacgaaaaaatcggcgtaggcttcaacgcagcaaccggcgaatgggtaaacatgatcgaaaaaggtatcgttgacccgacaaaagttacacgttctgcacttcaaaatgcagcttctgtagcagcaatgctcctgacaactgaagcggttgtcgctgacaaaccggaagaaaacgccggcggcgcaggaatgcctgacatgggcggaatgggcggtatgggcggaatgatgtaa

SEQ ID NO: 16 - DNA, 1547 bp, Bacillus subtilis; identical to SEQ ID NO: 1

SEQ ID NO: 17 - DNA, 1197 bp, Bacillus subtilis; identical to SEQ ID NO: 2

SEQ ID NO: 18 - DNA, 1923 bp, Bacillus subtilis; identical to SEQ ID NO: 3

SEQ ID NO: 19 - DNA, 3582 bp, Bacillus subtilis; identical to SEQ ID NO: 4

SEQ ID NO: 20 - DNA, 1632 bp, Bacillus subtilis; identical to SEQ ID NO: 5